European Patent Application EP 4 372 104 A1, published May 22, 2024. Title: Composition for In-situ Detecting Microbial Contamination and Uses Thereof. Applicant: BioNano Health Guard Research Center. The sequence listing filed with the application follows.

SEQUENCE LISTING (5 sequences)

SEQ ID NO: 1 - DNA, 36 bp, Artificial Sequence
  DNA1
atcaccctccccgcacctaaagggtgcggggagggt

SEQ ID NO: 2 - DNA, 32 bp, Artificial Sequence
  DNA2
accctccccgcaccctattggtgcggggaggg

SEQ ID NO: 3 - DNA, 32 bp, Artificial Sequence; identical to SEQ ID NO: 2
  DNA3

SEQ ID NO: 4 - DNA, 36 bp, Artificial Sequence; identical to SEQ ID NO: 1
  DNA4

SEQ ID NO: 5 - DNA, 35 bp, Artificial Sequence
  DNA5
tcgggacactgaaccctaaaggggttcagtgtccc